European Patent Application EP 4 772 162 A1, published July 8, 2026. Title: Composition for Improving Skin Condition Comprising Peptide As Active Ingredient. Applicant: CAREGEN CO., LTD. Application KR. The sequence listing filed with the application follows.

SEQUENCE LISTING (13 sequences)

SEQ ID NO: 1 - protein, 4 aa, synthetic construct
RLLN

SEQ ID NO: 2 - DNA, 20 bp, synthetic construct
  source 1..20: mol_type = other DNA
caccctcaagagcctgagtc

SEQ ID NO: 3 - DNA, 20 bp, synthetic construct
  source 1..20: mol_type = other DNA
agacggctgagtagggaaca

SEQ ID NO: 4 - DNA, 20 bp, synthetic construct
  source 1..20: mol_type = other DNA
ccaggaaccgagtacaccat

SEQ ID NO: 5 - DNA, 20 bp, synthetic construct
  source 1..20: mol_type = other DNA
atacccaggttgggtgatga

SEQ ID NO: 6 - DNA, 20 bp, synthetic construct
  source 1..20: mol_type = other DNA
gcaagacctggctttggact

SEQ ID NO: 7 - DNA, 21 bp, synthetic construct
  source 1..21: mol_type = other DNA
gggagtttctggttagggctg

SEQ ID NO: 8 - DNA, 20 bp, synthetic construct
  source 1..20: mol_type = other DNA
ccttcttgggtgctggaata

SEQ ID NO: 9 - DNA, 20 bp, synthetic construct
  source 1..20: mol_type = other DNA
acacgataagggaggctgtg

SEQ ID NO: 10 - DNA, 20 bp, synthetic construct
  source 1..20: mol_type = other DNA
tcagtggctggaacagtgag

SEQ ID NO: 11 - DNA, 20 bp, synthetic construct
  source 1..20: mol_type = other DNA
tctggcatgtcccactatca

SEQ ID NO: 12 - DNA, 20 bp, synthetic construct
  source 1..20: mol_type = other DNA
ggagccaaaagggtcatcat

SEQ ID NO: 13 - DNA, 20 bp, synthetic construct
  source 1..20: mol_type = other DNA
gtgatggcatggactgtggt